European Patent Specification EP 4 030 166 B1, published June 28, 2023. Title: HIGH-THROUGHPUT AND HIGHLY MULTIPLEXED IMAGING WITH PROGRAMMABLE NUCLEIC ACID PROBES. Applicant: President and Fellows of Harvard College. Application EP15762370.3. The sequence listing filed with the application follows.

SEQUENCE LISTING (11 sequences)

SEQ ID NO: 1 - DNA, 11 bp, Artificial Sequence
  Synthetic Polynucleotide
catctaaagcc

SEQ ID NO: 2 - DNA, 11 bp, Artificial Sequence
  Synthetic Polynucleotide
gaatttcctcg

SEQ ID NO: 3 - DNA, 11 bp, Artificial Sequence
  Synthetic Polynucleotide
gtttaattgcg

SEQ ID NO: 4 - DNA, 11 bp, Artificial Sequence
  Synthetic Polynucleotide
acaattcttcg

SEQ ID NO: 5 - DNA, 11 bp, Artificial Sequence
  Synthetic Polynucleotide
tttcttgcttc

SEQ ID NO: 6 - DNA, 11 bp, Artificial Sequence
  Synthetic Polynucleotide
gcattgttact

SEQ ID NO: 7 - DNA, 11 bp, Artificial Sequence
  Synthetic Polynucleotide
atatacaagcg

SEQ ID NO: 8 - DNA, 11 bp, Artificial Sequence
  Synthetic Polynucleotide
gctgtctattg

SEQ ID NO: 9 - DNA, 11 bp, Artificial Sequence
  Synthetic Polynucleotide
tctttatgctg

SEQ ID NO: 10 - DNA, 11 bp, Artificial Sequence
  Synthetic Polynucleotide
caatctcatcc

SEQ ID NO: 11 - DNA, 11 bp, Artificial Sequence
  Reverse complementary strand of SEQ ID NO: 1
ggctttagatg